European Patent Application EP 4 624 574 A1, published October 1, 2025. Title: UTR MOLECULE FOR INCREASING PROTEIN EXPRESSION LEVEL. Applicant: 苏州艾博生物科技有限公司. Application CN. The sequence listing filed with the application follows.

SEQUENCE LISTING (39 sequences)

SEQ ID NO: 1-2 - skipped (2 entries)

SEQ ID NO: 3 - DNA, 53 bp, synthetic construct
  source 1..53: mol_type = other DNA
gattgcttatagaccggaagccgggaccttaattctctttcccatcttgcaag

SEQ ID NO: 4 - DNA, 59 bp, synthetic construct
  source 1..59: mol_type = other DNA
ctgaactgggttaggtgccgctgttgctgctcgtgttgaatctagaaccgtagccagac

SEQ ID NO: 5 - DNA, 82 bp, synthetic construct
  source 1..82: mol_type = other DNA
aaaattttgcagggtaaattagcctgtctgggtctgagctctttattcttggatacgttggagatcggaaagatattaagat

SEQ ID NO: 6 - DNA, 73 bp, synthetic construct
  source 1..73: mol_type = other DNA
agtatattagtgctaatttccctccgtttgtcctagcttttctcttctgtcaaccccacacgcctttggcaca

SEQ ID NO: 7 - DNA, 71 bp, synthetic construct
  source 1..71: mol_type = other DNA
cggcgcgccgggcttcgcgctccggtacttcctatttaacagacattgtgtggtgggctggcacaatcgca

SEQ ID NO: 8 - DNA, 80 bp, synthetic construct
  source 1..80: mol_type = other DNA
ttcctgtcccgctcggctccaggccctgcgtgtcccagggactgcggccggggcggggtggggctctcccctggccagga

SEQ ID NO: 9 - DNA, 22 bp, synthetic construct
  source 1..22: mol_type = other DNA
ttctcccccaggctcactcacc

SEQ ID NO: 10 - DNA, 56 bp, synthetic construct
  source 1..56: mol_type = other DNA
gccaggccggccaggcctgcgccgccgccgccgccgccgtcgccgccgcgccgacc

SEQ ID NO: 11 - DNA, 81 bp, synthetic construct
  source 1..81: mol_type = other DNA
aacgggggcgcgcggtcgggggcaggttgggccggaagaggggtccgggccggcactgaggcgggaagggggtcggttgag

SEQ ID NO: 12 - DNA, 55 bp, synthetic construct
  source 1..55: mol_type = other DNA
agttccctatcactctctttaatcactactcacagtaacctcaactcctgccaca

SEQ ID NO: 13 - DNA, 30 bp, synthetic construct
  source 1..30: mol_type = other DNA
gctggttttggtgatttttgtctgattgca

SEQ ID NO: 14 - DNA, 69 bp, synthetic construct
  source 1..69: mol_type = other DNA
gcctcttccccctcccgcgcgcccgcccgccgcctgccgccgccgccgccgccgccggagctctgtagt

SEQ ID NO: 15 - DNA, 71 bp, synthetic construct
  source 1..71: mol_type = other DNA
tgtgagttcattcctccctgctcagattcttcagctcctcgtggttggtttattcaattggttgtttcatt

SEQ ID NO: 16 - DNA, 74 bp, synthetic construct
  source 1..74: mol_type = other DNA
ctccttccctcgtcctgggtcccggggtcctgggtacgtttggctagcctgctctggcggtgcagaggggcagg

SEQ ID NO: 17 - DNA, 53 bp, synthetic construct
  source 1..53: mol_type = other DNA
attttgtttttgtgtttttgcagggaggagctcttcctgcaggcgtggaaacc

SEQ ID NO: 18 - skipped

SEQ ID NO: 19 - DNA, 70 bp, synthetic construct
  source 1..70: mol_type = other DNA
attaaggagaaaaagtaggaggaggaggagaaagagtgctttgcccagggtgtgactgaagaaatatcaa

SEQ ID NO: 20 - DNA, 39 bp, synthetic construct
  source 1..39: mol_type = other DNA
gaaataagagagaaaagaagagtaagaagaaatataaga

SEQ ID NO: 21 - DNA, 46 bp, synthetic construct
  source 1..46: mol_type = other DNA
gaataaactagtattcttctggtccccacagactcagagagaaccc

SEQ ID NO: 22 - DNA, 59 bp, synthetic construct
  source 1..59: mol_type = other DNA
aagcttagcttgcttgttctttttgcagaagctcagaataaacgctcaactttggcgcc

SEQ ID NO: 23 - DNA, 113 bp, synthetic construct
  source 1..113: mol_type = other DNA
taggctggagcctcggtggccatgcttcttgccccttgggcctccccccagcccctcctccccttcctgcacccgtacccccgtggtctttgaataaagtctgagtgggcggc

SEQ ID NO: 24 - DNA, 132 bp, synthetic construct
  source 1..132: mol_type = other DNA
gctggagcctcggtggccatgcttcttgccccttgggcctccccccagcccctcctccccttcctgcacccgtaccccccaaacaccattgtcacactccagtggtctttgaataaagtctgagtgggcggc

SEQ ID NO: 25 - DNA, 289 bp, synthetic construct
  source 1..289: mol_type = other DNA
ctggtactgcatgcacgcaatgctagctgcccctttcccgtcctgggtaccccgagtctcccccgacctcgggtcccaggtatgctcccacctccacctgccccactcaccacctctgctagttccagacacctcccaagcacgcagcaatgcagctcaaaacgcttagcctagccacacccccacgggaaacagcagtgattaacctttagcaataaacgaaagtttaactaagctatactaaccccagggttggtcaatttcgtgccagccacaccctggagctagc

SEQ ID NO: 26 - DNA, 100 bp, synthetic construct
  source 1..100: mol_type = other DNA
ctgcctctcgctcctcaacccctcccctccatccctggccccctccctggatgacattaaagaagggttgagctggtccctgcctgcatgtgactgtaaa

SEQ ID NO: 27 - DNA, 897 bp, synthetic construct
  source 1..897: mol_type = other DNA
ataaaatgagaaaggtatgtttttcttttttaaaaaagctgctgttggatctagaaggtgaagaatttttttatgtatatatagacatatctatataaattgtctggctgaggcagggccttcagctatcatttggttaataaatacattttagtatttgcatttcctactgcctgcagagtttcaggtgcttgttgtgtgaaagttctgtagatgtgtgcaaatttaacgaaatgaaattgtatgtgtaaaaatgtacgatttttcactgtgcaactgtaaattataaataaaaaatatttttgctattcatggagtgtaatatttatgcacaccatcaaatagtttctgtactttttattgggtaaaaatggaattgaacagcaacctcaacataagattttttttctagtagcctcccactgattaaagaagcaagtttgaggtttcatccttcaaaagggggttccgagagagcaccgtagggcttttctcaaatagaaaagccagattttgaaaaaattttaaagataaaataggacatattttgcagatatatatatatatatacacaaacacatctccaggtatagagaaccatccagatgttcacttttgaaaatatctaatgatgcaaagttttattcttgaacttggacactgatgccatcaaacaattaacaaatatatttaagtactaaaggtgattttttttttaaagactttttcaaattgtcaaatgatttaatgcagatgaacatatttctattttaagtaacgggaatctgtaagaatgtttgcttgagatatggttaacttttttcttttgttggttttgacttagatggacaccatgagatgttaatattcatacatgtaataaatagaatgatgaag

SEQ ID NO: 28 - DNA, 122 bp, synthetic construct
  source 1..122: mol_type = other DNA
tcctttaagggagtgaggtgctgaggcctggtggcagaggcagccctggctcccccatggccactgtgtcctgctgggaaggagggcctggctccacgacccacctctgccggcctggggct

SEQ ID NO: 29 - DNA, 129 bp, synthetic construct
  source 1..129: mol_type = other DNA
cacccaggcctggagaagatgagacacctgggcccatctggctgctggagattcagtctcagttttatttctctgtggcactcactgcttctggaggggagactgttaataaaagatttgggaaccccc

SEQ ID NO: 30 - DNA, 264 bp, synthetic construct
  source 1..264: mol_type = other DNA
gcagctggggtgcctccctcgggtgtccagcaagcactggggagtcccccttagggctggctttgagatagatcctgatgtcagcctgtttcacagatgagacaatggaggctttgatcgcttgcccagggccacgtccagtgagtggtacagcttggactcaaacccaagtctgtgtgactccaacatgtcacacttcctcacgtgaaaagcctcatatgaggctgggcacagtgacttgtgcctgtaatcccagcactttgg

SEQ ID NO: 31 - DNA, 161 bp, synthetic construct
  source 1..161: mol_type = other DNA
tgttctgccaggaacactgcttcctgccaggtacccacagaccatgggagcttaggttctgtgtgtctggaatgttttctgctgcttctctgctcacatggttggggggatgcaggggttgtgagggaaggcactgcttattgccaccttccagtgaatgc

SEQ ID NO: 32 - DNA, 660 bp, synthetic construct
  source 1..660: mol_type = other DNA
ttagggagtctgccctttttctgtgccctgggacctgagcatgtgggagcagggcagatgggtggcaggaggccaggggttggatcatgttccccccaaatgctgggaagcaataagcctcctcctccccccaccatttctctggagattaggacttattctcacagctggaggaagctcaacaactttcctgaggacaatgattgtttgaaaggcttgttttgtaaggaagccaggaggaatatatgagtttgatgagctaaaacagttcctcatttggtctagttttcgggccaggggagtaagtgaaattcacttctctataagaataagcccatccatctcttttattcatgaacagagacagaaagagtgcttggcatggcatgcctccgagggaggctgtgggaggaggccaagctggcaggctcgggttctttgcccttgctagcgcccaggtcagagggaaaaggaatgtactcgtacccttccctcaccaccttgtaggtccccaggtaccaggtgcccagggaagaaggccttcacaatgatccccccagctcagaacagcccctgcacacccagtaaccggcatctggcttctccttagcttagtgcagctgtggattctgggaaagtggcctctctaatctgaacttg

SEQ ID NO: 33 - DNA, 192 bp, synthetic construct
  source 1..192: mol_type = other DNA
gccaacccagacacagtgcggtaccagaattgccttagaagataccagaaggtgcggtctagggaccagtgaataagaagaccccacttcaacttcccctcgaagacgttgtgcctcacagcgaggcctacaagggatgggaacttttatttcaaaataaatactaccgaggctgtgatcaggctcaccttg

SEQ ID NO: 34 - DNA, 257 bp, synthetic construct
  source 1..257: mol_type = other DNA
agggggtggcagggcgggtcatggagctttcgcctgggtgctgttggttgcttggttggctggtggtttgggcagggggagttaggagctggcaggagtggggctgcatttttgaggcctttgggcatgatggtgaaatgtgtagactcgggtactctgcccaaccccatgggaagtgtgttggctttcaaccagcctgcgtgtttctccactgctcagctcttctggagaggttgtcatcattgtatttgtggttt

SEQ ID NO: 35 - DNA, 45 bp, synthetic construct
  source 1..45: mol_type = other DNA
gcatcctgctgccttcccacaacattaaactctccttcctcagtg

SEQ ID NO: 36 - DNA, 155 bp, synthetic construct
  source 1..155: mol_type = other DNA
gagaacagtcaggcagggagcccttctccccacagagctttcaggagcagacagtggcctccccttcccctccctgccccaggacttaaagagcaatagtttgccccttttggaatgatctctgaatatataaaacacacacacaaagagcaata

SEQ ID NO: 37 - DNA, 21 bp, synthetic construct
  source 1..21: mol_type = other DNA
taatacgactcactatagggg

SEQ ID NO: 38 - DNA, 585 bp, synthetic construct
  source 1..585: mol_type = other DNA
atgggggtgcacgaatgtcctgcctggctgtggcttctcctgtccctgctgtcgctccctctgggcctcccagtcctgggcgccccaccacgcctcatctgtgacagccgagtcctggagaggtacctcttggaggccaaggaggccgagaatatcacgacgggctgtgctgaacactgcagcttgaatgagaatatcactgtcccagacaccaaagttaatttctatgcctggaagaggatggaggtcgggcagcaggccgtagaagtctggcagggcctggccctgctgtcggaagctgtcctgcggggccaggccctgttggtcaactcttcccagccgtgggagcccctgcagctgcatgtggataaagccgtcagtggccttcgcagcctcaccactctgcttcgggctctgggagcccagaaggaagccatctcccctccagatgcggcctcagctgctccactccgaacaatcactgctgacactttccgcaaactcttccgagtctactccaatttcctccggggaaagctgaagctgtacacaggggaggcctgcaggacaggggacagatgataa

SEQ ID NO: 39 - DNA, 723 bp, synthetic construct
  source 1..723: mol_type = other DNA
atggtgagcaagggcgaggagctgttcaccggggtggtgcccatcctggtcgagctggacggcgacgtaaacggccacaagttcagcgtgtccggcgagggcgagggcgatgccacctacggcaagctgaccctgaagttcatctgcaccaccggcaagctgcccgtgccctggcccaccctcgtgaccaccctgacctacggcgtgcagtgcttcagccgctaccccgaccacatgaagcagcacgacttcttcaagtccgccatgcccgaaggctacgtccaggagcgcaccatcttcttcaaggacgacggcaactacaagacccgcgccgaggtgaagttcgagggcgacaccctggtgaaccgcatcgagctgaagggcatcgacttcaaggaggacggcaacatcctggggcacaagctggagtacaactacaacagccacaacgtctatatcatggccgacaagcagaagaacggcatcaaggtgaacttcaagatccgccacaacatcgaggacggcagcgtgcagctcgccgaccactaccagcagaacacccccatcggcgacggccccgtgctgctgcccgacaaccactacctgagcacccagtccgccctgagcaaagaccccaacgagaagcgcgatcacatggtcctgctggagttcgtgaccgccgccgggatcactctcggcatggacgagctgtacaagtgataa